European Patent Application EP 4 324 916 A1, published February 21, 2024. Title: A method of activating and proliferating exhausted CD8 T cells, CD8 T cells with enhanced activity prepared by the same, and use thereof. Applicant: Seoul National University R&DB Foundation MEDGENE THERAPEUTICS, INC. The sequence listing filed with the application follows.

SEQUENCE LISTING (18 sequences)

SEQ ID NO: 1 - DNA, 1452 bp, Mus msculus
atgaggcagccacctggcgagtctgacatggctgtcagcgacgctctgctcccgtccttctccacgttcgcgtccggcccggcgggaagggagaagacactgcgtccagcaggtgccccgactaaccgttggcgtgaggaactctctcacatgaagcgacttcccccacttcccggccgcccctacgacctggcggcgacggtggccacagacctggagagtggcggagctggtgcagcttgcagcagtaacaacccggccctcctagcccggagggagaccgaggagttcaacgacctcctggacctagactttatcctttccaactcgctaacccaccaggaatcggtggccgccaccgtgaccacctcggcgtcagcttcatcctcgtcttccccggcgagcagcggccctgccagcgcgccctccacctgcagcttcagctatccgatccgggccgggggtgacccgggcgtggctgccagcaacacaggtggagggctcctctacagccgagaatctgcgccacctcccacggcccccttcaacctggcggacatcaatgacgtgagcccctcgggcggcttcgtggctgagctcctgcggccggagttggacccagtatacattccgccacagcagcctcagccgccaggtggcgggctgatgggcaagtttgtgctgaaggcgtctctgaccacccctggcagcgagtacagcagcccttcggtcatcagtgttagcaaaggaagcccagacggcagccaccccgtggtagtggcgccctacagcggtggcccgccgcgcatgtgccccaagattaagcaagaggcggtcccgtcctgcacggtcagccggtccctagaggcccatttgagcgctggaccccagctcagcaacggccaccggcccaacacacacgacttccccctggggcggcagctccccaccaggactacccctacactgagtcccgaggaactgctgaacagcagggactgtcaccctggcctgcctcttcccccaggattccatccccatccggggcccaactaccctcctttcctgccagaccagatgcagtcacaagtcccctctctccattatcaagagctcatgccaccgggttcctgcctgccagaggagcccaagccaaagaggggaagaaggtcgtggccccggaaaagaacagccacccacacttgtgactatgcaggctgtggcaaaacctataccaagagttctcatctcaaggcacacctgcgaactcacacaggcgagaaaccttaccactgtgactgggacggctgtgggtggaaattcgcccgctccgatgaactgaccaggcactaccgcaaacacacagggcaccggccctttcagtgccagaagtgtgacagggccttttccaggtcggaccaccttgccttacacatgaagaggcacttttaa

SEQ ID NO: 2 - DNA, 29 bp, Artificial Sequence
  Forward primer coloning klf4 gene
agatctaccatgaggcagccacctggcga

SEQ ID NO: 3 - DNA, 36 bp, Artificial Sequence
  Reverse primer for cloning klf4 gene
gaattcttaaaagtgcctcttcatgtgtaaggcaag

SEQ ID NO: 4 - protein, 483 aa, Mus musulus
MRQPPGESDMAVSDALLPSFSTFASGPAGREKTLRPAGAPTNRWREELSHMKRLPPLPGRPYDLAATVATDLESGGAGAACSSNNPALLARRETEEFNDLLDLDFILSNSLTHQESVAATVTTSASASSSSSPASSGPASAPSTCSFSYPIRAGGDPGVAASNTGGGLLYSRESAPPPTAPFNLADINDVSPSGGFVAELLRPELDPVYIPPQQPQPPGGGLMGKFVLKASLTTPGSEYSSPSVISVSKGSPDGSHPVVVAPYSGGPPRMCPKIKQEAVPSCTVSRSLEAHLSAGPQLSNGHRPNTHDFPLGRQLPTRTTPTLSPEELLNSRDCHPGLPLPPGFHPHPGPNYPPFLPDQMQSQVPSLHYQELMPPGSCLPEEPKPKRGRRSWPRKRTATHTCDYAGCGKTYTKSSHLKAHLRTHTGEKPYHCDWDGCGWKFARSDELTRHYRKHTGHRPFQCQKCDRAFSRSDHLALHMKRHF

SEQ ID NO: 5 - protein, 504 aa, Homo sapiens
MAVSDALLPSFSTFASGPAGREKTLRQAGAPNNRWREELSHMKRLPPVLPGRPYDLAAATVATDLESGGAGAACGGSNLAPLPRRETEEFNDLLDLDFILSNSLTHPPESVAATVSSSASASSSSSPSSSGPASAPSTCSFTYPIRAGNDPGVAPGGTGGGLLYGRESAPPPTAPFNLADINDVSPSGGFVAELLRPELDPVYIPPQQPQPPGGGLMGKFVLKASLSAPGSEYGSPSVISVSKGSPDGSHPVVVAPYNGGPPRTCPKIKQEAVSSCTHLGAGPPLSNGHRPAAHDFPLGRQLPSRTTPTLGLEEVLSSRDCHPALPLPPGFHPHPGPNYPSFLPDQMQPQVPPLHYQGQSRGFVARAGEPCVCWPHFGTHGMMLTPPSSPLELMPPGSCMPEEPKPKRGRRSWPRKRTATHTCDYAGCGKTYTKSSHLKAHLRTHTGEKPYHCDWDGCGWKFARSDELTRHYRKHTGHRPFQCQKCDRAFSRSDHLALHMKRHF

SEQ ID NO: 6 - DNA, 1515 bp, Homo sapiens
atggctgtcagcgacgcgctgctcccatctttctccacgttcgcgtctggcccggcgggaagggagaagacactgcgtcaagcaggtgccccgaataaccgctggcgggaggagctctcccacatgaagcgacttcccccagtgcttcccggccgcccctatgacctggcggcggcgaccgtggccacagacctggagagcggcggagccggtgcggcttgcggcggtagcaacctggcgcccctacctcggagagagaccgaggagttcaacgatctcctggacctggactttattctctccaattcgctgacccatcctccggagtcagtggccgccaccgtgtcctcgtcagcgtcagcctcctcttcgtcgtcgccgtcgagcagcggccctgccagcgcgccctccacctgcagcttcacctatccgatccgggccgggaacgacccgggcgtggcgccgggcggcacgggcggaggcctcctctatggcagggagtccgctccccctccgacggctcccttcaacctggcggacatcaacgacgtgagcccctcgggcggcttcgtggccgagctcctgcggccagaattggacccggtgtacattccgccgcagcagccgcagccgccaggtggcgggctgatgggcaagttcgtgctgaaggcgtcgctgagcgcccctggcagcgagtacggcagcccgtcggtcatcagcgtcagcaaaggcagccctgacggcagccacccggtggtggtggcgccctacaacggcgggccgccgcgcacgtgccccaagatcaagcaggaggcggtctcttcgtgcacccacttgggcgctggaccccctctcagcaatggccaccggccggctgcacacgacttccccctggggcggcagctccccagcaggactaccccgaccctgggtcttgaggaagtgctgagcagcagggactgtcaccctgccctgccgcttcctcccggcttccatccccacccggggcccaattacccatccttcctgcccgatcagatgcagccgcaagtcccgccgctccattaccaaggtcagtcccggggatttgtagctcgggctggggagccctgtgtgtgctggccccacttcgggacacacgggatgatgctcaccccaccttcttcacccctagagctcatgccacccggttcctgcatgccagaggagcccaagccaaagaggggaagacgatcgtggccccggaaaaggaccgccacccacacttgtgattacgcgggctgcggcaaaacctacacaaagagttcccatctcaaggcacacctgcgaacccacacaggtgagaaaccttaccactgtgactgggacggctgtggatggaaattcgcccgctcagatgaactgaccaggcactaccgtaaacacacggggcaccgcccgttccagtgccaaaaatgcgaccgagcattttccaggtcggaccacctcgccttacacatgaagaggcatttttaa

SEQ ID NO: 7 - DNA, 19 bp, Artificial Sequence
  Forward primer for detecting klf4 gene
gtgccccgactaaccgttg

SEQ ID NO: 8 - DNA, 20 bp, Artificial Sequence
  Reverse primer for detecting klf4 gene
gtcgttgaactcctcggtct

SEQ ID NO: 9 - DNA, 20 bp, Artificial Sequence
  Forward primer for detecting tox gene
caactcaaagccgtcagtat

SEQ ID NO: 10 - DNA, 20 bp, Artificial Sequence
  Reverse primer for detecting tox gene
gctgaggagtcattcctggt

SEQ ID NO: 11 - protein, 254 aa, Artificial Sequence
  anti-EpCAM scFv
DIQMTQSPSSLSASVGDRVTITCRSTKSLLHSNGITYLYWYQQKPGKAPKLLIYQMSNLASGVPSRFSSSGSGTDFTLTISSLQPEDFATYYCAQNLEIPRTFGQGTKVELKRATPSHNSHQVPSAGGPTANSGTSGSEVQLVQSGPGLVQPGGSVRISCAASGYTFTNYGMNWVKQAPGKGLEWMGWINTYTGESTYADSFKGRFTFSLDTSASAAYLQINSLRAEDTAVYYCARFAIKGDYWGQGTLLTVSS

SEQ ID NO: 12 - protein, 45 aa, Artificial Sequence
  CD8 alpha hinge
TTTPAPRPPTPAPTIASQPLSLRPEACRPAAGGAVHTRGLDFACD

SEQ ID NO: 13 - protein, 27 aa, Artificial Sequence
  CD28 transmembrane domain
FWVLVVVGGVLACYSLLVTVAFIIFWV

SEQ ID NO: 14 - protein, 112 aa, Artificial Sequence
  CD28 (CD
RVKFSRSADAPAYQQGQNQLYNELNLGRREEYDVLDKRRGRDPEMGGKPRRKNPQEGLYNELQKDKMAEAYSEIGMKGERRRGKGHDGLYQGLSTATKDTYDALHMQALPPR

SEQ ID NO: 15 - protein, 112 aa, Artificial Sequence; identical to SEQ ID NO: 14
  CD3 zeta ICD

SEQ ID NO: 16 - protein, 240 aa, Artificial Sequence
  anti-Trop-2 scFv
QVQLQQSGSELKKPGASVKVSCKASGYTFTNYGMNWVKQAPGQGLKWMGWINTYTGEPTYTDDFKGRFAFSLDTSVSTAYLQISSLKADDTAVYFCARGGFGSSYWYFDVWGQGSLVTVSSGGGGSGGGGSGGGGSDIQLTQSPSSLSASVGDRVSITCKASQDVSIAVAWYQQKPGKAPKLLIYSASYRYTGVPDRFSGSGSGTDFTLTISSLQPEDFAVYYCQQHYITPLTFGAGTKV

SEQ ID NO: 17 - protein, 243 aa, Artificial Sequence
  anti-CEACAM6 scFv
QVQLQESGGGVVQPGRSLRLSCSSSGFALTDYYMSWVRQAPGKGLEWLGFIANKANGHTTDYSPSVKGRFTISRDNSKNTLFLQMDSLRPEDTGVYFCARDMGIRWNFDVWGQGTPVTVSSGGGGSGGGGSGGGGSDIQLTQSPSSLSASVGDRVTMTCSASSRVSYIHWYQQKPGKAPKRWIYGTSTLASGVPARFSGSGSGTDFTFTISSLQPEDIATYYCQQWSYNPPTFGQGTKVEIKR

SEQ ID NO: 18 - protein, 241 aa, Artificial Sequence
  anti-CEACAM5 scFv
EVQLVESGGGVVQPGRSLRLSCSASGFDFTTYWMSWVRQAPGKGLEWIGEIHPDSSTINYAPSLKDRFTISRDNAKNTLFLQMDSLRPEDTGVYFCASLYFGFPWFAYWGQGTPVTVSSGGGGSGGGGSGGGGSDIQLTQSPSSLSASVGDRVTITCKASQDVGTSVAWYQQKPGKAPKLLIYWTSTRHTGVPSRFSGSGSGTDFTFTISSLQPEDIATYYCQQYSLYRSFGQGTKVEIKR